European Patent Specification EP 3 990 434 B1, published June 25, 2025. Title: COMPOUNDS HAVING ANTIMALARIAL ACTIVITY. Applicant: Nanyang Technological University. The sequence listing filed with the application follows.

SEQUENCE LISTING (3 sequences)

SEQ ID NO: 1 - DNA, 54 bp, Artificial
  oligonucleotide primer
tgacactatagaatactcgcggccgctgcatctaccttcatcagatgcatcaac

SEQ ID NO: 2 - DNA, 57 bp, Artificial
  oligonucleotide primer
caccagcagcagcacctctagcacgcgtttctttggtttcccatttccaaacttttg

SEQ ID NO: 3 - protein, 10 aa, Artificial
  peptide substrate
HKRHSFRMRG